European Patent Application EP 4 159 869 A1, published April 5, 2023. Title: PRODUCTION OF BACTERIAL NANOCELLULOSE. Applicant: Consejo Superior de Investigaciones Científicas (CSIC). The sequence listing filed with the application follows.

SEQUENCE LISTING (1 sequence)

SEQ ID NO: 1 - DNA, 1214 bp, Artificial Sequence
  Deletion in gene bcsA
tcggagaacgagatgttctacggcatcatccagcgcggcctcgacaagtgggacgccgccttcttctgcggttcggcggcggtgctcagccggcgcgccctgggcgaaagcaacggcttcagcggcgtcaccatcaccgaggactgcgagaccgcgctcgagctgcactcgcgcggctggcactcgatctatgtcgacaagccgatgatcgccggcctccagccggacagctatgccagcttcatcgtccagcgctcgcgctgggcgcagggcatgatgcagatcctgcgcttccacttcccgccgggcaagcgcggcctcaccctggcgcagcgcctgtgctactgctccagcaccttcttctggctgttcccctattcgcggctgatgttcctcatctcgccgctgttctacctgttcttctcgctggagatcttcaacgcctccggcgccgagttcctcgcctacaccaccacctatatgctggtgaacctgctgatgcagaactacctctatggccgctaccgctggccatggatctccgagctctacgaatacatccagtcgatctacctgttccccgcgctcgtggcggtgctggccaatccgcgcaagccgaccttcaaggtgacgtcgaagggcgagcacatggacgagggccatgtgtcggagatcggcccgcccttcttcatcattttcggcatcctcgtcctcggcgtggtgctgaccatctggcgcctgctgaccgagccgttcaaccatgacgtcatcatcgtcgtcggcggctggaacctcctgaacctgctgctcgccggctgcgcgctgggcgtcgtctccgagcgccgcaaccgccgccgcacgcaccgcgtcgacctgctgcgccggggcgagatcgtcatcaacggcgtcgcctatccggccgccatcgaggacggctcgctcggcggcgcgcgggtgcggctggcggccaacgtgacggtgccggagttcgagcgcggcacggtgggcctgctgcgcttccggccgctggccaccaacatcccgatcgacctgctcccggtcacgatccgcaatgtcgagcgcggcgccgagggcgcgctgctcggctgccagttccacccggatcagccgctgcactaccgcctgatcgccgacctgatcttcgccaattccgacgaatggcagaaattcctggattcgcgccggaagaaccc